European Patent Specification EP 3 814 354 B1, published November 8, 2023. Title: PURINE COMPOUNDS AND METHOD FOR THE TREATMENT OF CANCER. Applicant: THE ROYAL INSTITUTION FOR THE ADVANCEMENT OF LEARNING/MCGILL UNIVERSITY ALAOUI-JAMALI , Moulay A BIJIAN, Krikor WERNIC, Dominik. The sequence listing filed with the application follows.

SEQUENCE LISTING (12 sequences)

SEQ ID NO: 1 - DNA, 29 bp, Artificial Sequence
  Sense primer sequence for Aurora A
cgggatccatggaccgatctaaagaaaac

SEQ ID NO: 2 - DNA, 30 bp, Artificial Sequence
  Antisense primer sequence for Aurora A
ccgctcgagagactgtttgctagctgattc

SEQ ID NO: 3 - DNA, 27 bp, Artificial Sequence
  Sense primer sequence for Aurora B
cgggatccatgagccgctccaatgtcc

SEQ ID NO: 4 - DNA, 27 bp, Artificial Sequence
  Antisense primer sequence for Aurora B
ccgctcgagggcgacagattgaagggc

SEQ ID NO: 5 - RNA, 21 nt, Artificial Sequence
  non-targeted siRNA sense sequence
  modified_base (20)...(21): deoxythymidine
uucuccgaacgugucacgunn

SEQ ID NO: 6 - RNA, 22 nt, Artificial Sequence
  non-targeted siRNA antisense sequence
  modified_base (21)...(22): deoxythymidine
acggugacacguucggagaann

SEQ ID NO: 7 - RNA, 24 nt, Artificial Sequence
  Beclin1 siRNA sense sequence
  modified_base (23)...(24): deoxythymidine
cucaaguucaugcugacgaauunn

SEQ ID NO: 8 - RNA, 24 nt, Artificial Sequence
  Beclin1 siRNA antisense sequence
  modified_base (23)...(24): deoxythymidine
uucgucagcaugaacuugaguunn

SEQ ID NO: 9 - RNA, 24 nt, Artificial Sequence
  Atg5 siRNA sense sequence
  modified_base (23)...(24): deoxythymidine
agauugaaggaucaacuauuuunn

SEQ ID NO: 10 - RNA, 24 nt, Artificial Sequence
  Atg5 siRNA antisense sequence
  modified_base (23)...(24): deoxythymidine
aauaguugauccuucaaucuuunn

SEQ ID NO: 11 - RNA, 24 nt, Artificial Sequence
  Atg7 siRNA sense sequence
  modified_base (23)...(24): deoxythymidine
gccugcugaggagcucuccauunn

SEQ ID NO: 12 - RNA, 22 nt, Artificial Sequence
  Atg7 siRNA antisense sequence
uggagagcuccucagcaggcuu